European Patent Specification EP 3 630 195 B1, published July 8, 2026. Title: AN INSULIN-LIKE GROWTH FACTOR-CHEMOTHERAPEPUTIC CONJUGATE FOR TREATING MYELODYSPLASTIC SYNDROME. Applicant: IGF Oncology, LLC McTavish, Hugh Dudek, Arkadiusz Z. The sequence listing filed with the application follows.

SEQUENCE LISTING (11 sequences)

SEQ ID NO: 1 - protein, 18 aa, Artificial
  Synthesized
MVKGKHHHHHHNGKGKSK

SEQ ID NO: 2 - protein, 88 aa, Artificial
  Synthesized
MVKGKHHHHHHNGKGKSKGPRTLCGAELVDALQFVCGDRGFYFNKPTGYGSSSRRAPQTGIVDECCFRSCDLRRLEMYCAPLKPAKSA

SEQ ID NO: 3 - protein, 70 aa, Homo sapiens
GPETLCGAELVDALQFVCGDRGFYFNKPTGYGSSSRRAPQTGIVDECCFRSCDLRRLEMYCAPLKPAKSA

SEQ ID NO: 4 - protein, 71 aa, Artificial
  Synthesized
FVNQHLCGSHLVEALYLVCGDRGFYFNKPTGYGSSSRRAPQTGIVDECCFRSCDLRRLEMYCAPLKPAKSA

SEQ ID NO: 5 - protein, 83 aa, Artificial
  Synthesized
MFPAMPLSSLFVNGPRTLCGALVDALQFVCGDRGFYFNKPTGYGSSSRRAPQTGIVDECCFRSCDLRRLEMYCAPLKPAKSEA

SEQ ID NO: 6 - protein, 70 aa, Artificial
  Synthesized
GPRTLCGAELVDALQFVCGDRGFYFNKPTGYGSSSRRAPQTGIVDECCFRSCDLRRLEMYCAPLKPAKSA

SEQ ID NO: 7 - protein, 67 aa, Artificial
  Synthesized
TLCGAELVDALQFVCGDRGFYFNKPTGYGSSSRRAPQTGIVDECCFRSCDLRRLEMYCAPLKPAKSA

SEQ ID NO: 8 - protein, 87 aa, Artificial
  Synthesized
MTSGHHHHHHSAGVNGFVNQHLCGSHLVEALYLVCGDRGFYFNKPTGYGSSSRRAPQTGIVDECCFRSCDLRRLEMYCAPLKPAKSA

SEQ ID NO: 9 - protein, 190 aa, Artificial
  Synthesized
MVKQIESKTAFQEALDAAGDKLVVVDFSATWCGHCKMIKPFFHSLSEKYSNVIFLEVDVDDSQDVASESEVKSMPTFQFFKKGQKVGEFSGANKEKLEATINELVGSKSGHHHHHHSAKGGPRTLCGAELVDALQFVCGDRGFYFNKPTGYGSSSRRAPQTGIVDECCFRSCDLRRLEMYCAPLKPAKSA

SEQ ID NO: 10 - protein, 191 aa, Artificial
  Synthesized
MVKQIESKTAFQEALDAAGDKLVVVDFSATWCGHCKMIKPFFHSLSEKYSNVIFLEVDVDDSQDVASESEVKSMPTFQFFKKGQKVGEFSGANKEKLEATINELVGSKSGHHHHHHSAKGFVNQHLCGSHLVEALYLVCGDRGFYFNKPTGYGSSSRRAPQTGIVDECCFRSCDLRRLEMYCAPLKPAKSA

SEQ ID NO: 11 - protein, 89 aa, Artificial
  Synthesized
MVKGKHHHHHHNGKGKSKFVNQHLCGSHLVEALYLVCGDRGFYFNKPTGYGSSSRRAPQTGIVDECCFRSCDLRRLEMYCAPLKPAKSA